European Patent Application EP 4 471 035 A1, published December 4, 2024. Title: PREPARATION METHOD FOR DRUG LINKER CONJUGATE. Applicant: MEDILINK THERAPEUTICS (SUZHOU) CO., LTD. The sequence listing filed with the application follows.

SEQUENCE LISTING (2 sequences)

SEQ ID NO: 1 - protein, 450 aa, Homo sapiens
EVQLLESGGGLVQPGGSLRLSCAASGFTFSSYAMNWVRQAPGKGLEWVSGISGSGGSTYYADSVQGRFTISRDNSKNTLYLQMNSLRAEDTAVYYCAKARSGYDYFFDYWGQGTLVTVSSASTKGPSVFPLAPSSKSTSGGTAALGCLVKDYFPEPVTVSWNSGALTSGVHTFPAVLQSSGLYSLSSVVTVPSSSLGTQTYICNVNHKPSNTKVDKKVEPKSCDKTHTCPPCPAPELLGGPSVFLFPPKPKDTLMISRTPEVTCVVVDVSHEDPEVKFNWYVDGVEVHNAKTKPREEQYNSTYRVVSVLTVLHQDWLNGKEYKCKVSNKALPAPIEKTISKAKGQPREPQVYTLPPSRDELTKNQVSLTCLVKGFYPSDIAVEWESNGQPENNYKTTPPVLDSDGSFFLYSKLTVDKSRWQQGNVFSCSVMHEALHNHYTQKSLSLSPGK

SEQ ID NO: 2 - protein, 215 aa, Homo sapiens
EIVLTQSPGTLSLSPGERATLSCRASQRISSSFLAWYQQKPGQAPSLLIYGASSRATGIPDRFSGSGSGTDFTLTISSLEPEDFAVFYCQQYSNSPLTFGGGTKVEIKRTVAAPSVFIFPPSDEQLKSGTASVVCLLNNFYPREAKVQWKVDNALQSGNSQESVTEQDSKDSTYSLSSTLTLSKADYEKHKVYACEVTHQGLSSPVTKSFNRGEC